European Patent Application EP 4 163 299 A1, published April 12, 2023. Title: MODIFIED-IgG ANTIBODIES THAT BIND TRANSFORMING GROWTH FACTOR-Beta1 WITH HIGH AFFINITY, AVIDITY AND SPECIFICITY. Applicant: Genzyme Corporation. The sequence listing filed with the application follows.

SEQUENCE LISTING (61 sequences)

SEQ ID NO: 1 - protein, 123 aa, Homo sapiens
EVQLVESGGGVVQPGRSLRLSCAASGFTFSSYGMHWVRQAPGKELEWVAVISYDGSIKYYADSVKGRFTISRDNSKNTLYLQMNSLRAEDTAVYYCARTGEYSGYDTDPQYSWGQGTTVTVSS

SEQ ID NO: 2 - protein, 123 aa, Homo sapiens
QVQLVESGGGVVQPGRSLRLSCAASGFTFSSYGMHWVRQAPGKELEWVAVISYDGSIKYYADSVKGRFTISRDNSKNTLYLQMNSLRAEDTAVYYCARTGEYSGYDTPASPDWGQGTTVTVSS

SEQ ID NO: 3 - protein, 107 aa, Homo sapiens
EIVLTQSPSSLSASVGDRVTITCRASQGIGDDLGWYQQKPGKAPILLIYGTSTLQSGVPSRFSGSGSGTDFTLTINSLQPEDFATYYCLQDSNYPLTFGGGTRLEIK

SEQ ID NO: 4 - protein, 107 aa, Homo sapiens
EIVLTQSPSSLSASVGDRVTITCRSSQGIGDDLGWYQQKPGKAPILLIYGTSTLQSGVPSRFSGSGSGTDFTLTINSLQPEDFATYYCLQDSNYPLTFGGGTRLEIK

SEQ ID NO: 5 - protein, 22 aa, Homo sapiens
PKSCDKTHTCPPCPAPELLGGP

SEQ ID NO: 6 - protein, 209 aa, Homo sapiens
SVFLFPPKPKDTLMISRTPEVTCVVVDVSHEDPEVKFNWYVDGVEVHNAKTKPREEQYNSTYRVVSVLTVLHQDWLNGKEYKCKVSNKALPAPIEKTISKAKGQPREPQVYTLPPSRDELTKNQVSLTCLVKGFYPSDIAVEWESNGQPENNYKTTPPVLDSDGSFFLYSKLTVDKSRWQQGNVFSCSVMHEALHNHYTQKSLSLSPGK

SEQ ID NO: 7 - protein, 5 aa, Homo sapiens
SYGMH

SEQ ID NO: 8 - protein, 17 aa, Homo sapiens
VISYDGSIKYYADSVKG

SEQ ID NO: 9 - protein, 14 aa, Homo sapiens
TGEYSGYDTSGVEL

SEQ ID NO: 10 - protein, 14 aa, Homo sapiens
TGEYSGYDTDPQYS

SEQ ID NO: 11 - protein, 14 aa, Homo sapiens
TGFYSGYDTPASPD

SEQ ID NO: 12 - protein, 11 aa, Homo sapiens
RASQGIGDDLG

SEQ ID NO: 13 - protein, 7 aa, Homo sapiens
GTSTLQS

SEQ ID NO: 14 - protein, 9 aa, Homo sapiens
LQDSNYPLT

SEQ ID NO: 15 - protein, 14 aa, Homo sapiens
  misc_feature (3)..(3): Xaa can be any naturally occurring amino acid
  misc_feature (10)..(14): Xaa can be any naturally occurring amino acid
TGXYSGYDTXXXXX

SEQ ID NO: 16 - protein, 213 aa, Homo sapiens
EWLTQSPSSLSASVGDRVTITCRASQGIGDDLGWYQQKPGKAPILLIYGTSTLQSGVPSRFSGSGSGTDFTLTINSLQPEDFATYYCLQDSNYPLTFGGGTRLEIKRTVAAPSVFIFPPSDEQLKSGTASVVCLLNNFYPREAKVQWKVDNALQSGNSQESVTEQDSKDSTYSLSSTLTLSKADYEKHKVYACEVTHQGLSSPVTKSFNRGEC

SEQ ID NO: 17 - protein, 450 aa, Homo sapiens
EVQLVESGGGVVQPGRSLRLSCAASGFTFSSYGMHWVRQAPGKELEWVAVISYDGSIKYYADSVKGRFTISRDNSKNTLYLQMNSLRAEDTAVYYCARTGEYSGYDTDPQYSWGQGTTVTVSSASTKGPSVFPLAPCSRSTSESTAALGCLVKDYFPEPVTVSWNSGALTSGVHTFPAVLQSSGLYSLSSVVTVPSSSLGTKTYTCNVDHKPSNTKVDKRVESKYGPPCPSCPAPEFLGGPSVFLFPPKPKDTLMISRTPEVTCVVVDVSQEDPEVQFNWYVDGVEVHNAKTKPREEQFNSTYRVVSVLTVLHQDWLNGKEYKCKVSNKGLPSSIEKTISKAKGQPREPQVYTLPPSQEEMTKNQVSLTCLVKGFYPSDIAVEWESNGQPENNYKTTPPVLDSDGSFFLYSRLTVDKSRWQEGNVFSCSVMHEALHNHYTQKSLSLSLGK

SEQ ID NO: 18 - protein, 450 aa, Homo sapiens
EVQLVESGGGVVQPGRSLRLSCAASGFTFSSYGMHWVRQAPGKELEWVAVISYDGSIKYYADSVKGRFTISRDNSKNTLYLQMNSLRAEDTAVYYCARTGEYSGYDTDPQYSWGQGTTVTVSSASTKGPSVFPLAPCSRSTSESTAALGCLVKDYFPEPVTVSWNSGALTSGVHTFPAVLQSSGLYSLSSVVTVPSSSLGTKTYTCNVDHKPSNTKVDKRVESKYGPPCPPCPAPEFLGGPSVFLFPPKPKDTLMISRTPEVTCVVVDVSQEDPEVQFNWYVDGVEVHNAKTKPREEQFNSTYRVVSVLTVLHQDWLNGKEYKCKVSNKGLPSSIEKTISKAKGQPREPQVYTLPPSQEEMTKNQVSLTCLVKGFYPSDIAVEWESNGQPENNYKTTPPVLDSDGSFFLYSRLTVDKSRWQEGNVFSCSVMHEALHNHYTQKSLSLSLGK

SEQ ID NO: 19 - protein, 245 aa, Homo sapiens
EVQLVESGGGVVQPGRSLRLSCAASGFTFSSYGMHWVRQAPGKELEWVAVISYDGSIKYYADSVKGRFTISRDNSKNTLYLQMNSLRAEDTAVYYCARTGEYSGYDTDPQYSWGQGTTVTVSSSGGGSGGGGSGGGGSEIVLTQSPSSLSASVGDRVTITCRSSQGIGDDLGWYQQKPGKAPILLIYGTSTLQSGVPSRFSGSGSGTDFTLTINSLQPEDFATYYCLQDSNYPLTFGGGTRLEIK

SEQ ID NO: 20 - protein, 112 aa, Homo sapiens
ALDTNYCFSSTEKNCCVRQLYIDFRKDLGWKWIHEPKGYHANFCLGPCPYIWSLDTQYSKVLALYNQHNPGASAAPCCVPQALEPLPIVYYVGRKPKVEQLSNMIVRSCKCS

SEQ ID NO: 21 - protein, 8 aa, Homo sapiens
LEIKRTVA

SEQ ID NO: 22 - protein, 9 aa, Homo sapiens
LEIKGRTVA

SEQ ID NO: 23 - protein, 10 aa, Homo sapiens
LEIKGGRTVA

SEQ ID NO: 24 - protein, 11 aa, Homo sapiens
LEIKGGSRTVA

SEQ ID NO: 25 - protein, 12 aa, Homo sapiens
LEIKGGGSRTVA

SEQ ID NO: 26 - protein, 13 aa, Homo sapiens
LEIKGGGGSRTVA

SEQ ID NO: 27 - DNA, 702 bp, Homo sapiens
atgggctggtcctgcatcatcctgtttctggtggccacagccaccggcgtgcacagcgagatcgtgctgacacagagccccagcagcctgtctgccagcgtgggcgacagagtgaccatcacctgtagagccagccagggcatcggcgacgacctgggatggtatcagcagaagcctggcaaggcccccatcctgctgatctacggcaccagcacactgcagagcggcgtgccctccagattttctggcagcggctccggcaccgacttcaccctgaccatcaacagcctgcagcccgaggacttcgccacctactactgtctgcaagacagcaactaccccctgaccttcggcggaggcacccggctggaaatcaagcgtacggtggccgctccttccgtgttcatcttccctccctccgacgagcagctgaagtccggcaccgcctccgtggtgtgtctgctgaacaacttctaccctcgggaggccaaggtgcagtggaaggtggacaacgccctgcagtccggcaactcccaggagtccgtcaccgagcaggactccaaggacagcacctactccctgtcctccaccctgaccctgtccaaggccgactacgagaagcacaaggtgtacgcctgtgaggtgacccaccagggcctgtccagccctgtgaccaagtccttcaaccggggcgagtgctga

SEQ ID NO: 28 - DNA, 31 bp, Homo sapiens
ggctggaaatcaagggccgtacggtggccgc

SEQ ID NO: 29 - DNA, 31 bp, Homo sapiens
gcggccaccgtacggcccttgatttccagcc

SEQ ID NO: 30 - DNA, 34 bp, Homo sapiens
ggctggaaatcaagggcggccgtacggtggccgc

SEQ ID NO: 31 - DNA, 34 bp, Homo sapiens
gcggccaccgtacggccgcccttgatttccagcc

SEQ ID NO: 32 - DNA, 37 bp, Homo sapiens
ggctggaaatcaagggcggcagccgtacggtggccgc

SEQ ID NO: 33 - DNA, 37 bp, Homo sapiens
gcggccaccgtacggctgccgcccttgatttccagcc

SEQ ID NO: 34 - DNA, 40 bp, Homo sapiens
ggctggaaatcaagggcggcggcagccgtacggtggccgc

SEQ ID NO: 35 - DNA, 40 bp, Homo sapiens
gcggccaccgtacggctgccgccgcccttgatttccagcc

SEQ ID NO: 36 - DNA, 43 bp, Homo sapiens
ggctggaaatcaagggcggcggcggcagccgtacggtggccgc

SEQ ID NO: 37 - DNA, 43 bp, Homo sapiens
gcggccaccgtacggctgccgccgccgcccttgatttccagcc

SEQ ID NO: 38 - protein, 214 aa, Homo sapiens
EIVLTQSPSSLSASVGDRVTITCRASQGIGDDLGWYQQKPGKAPILLIYGTSTLQSGVPSRFSGSGSGTDFTLTINSLQPEDFATYYCLQDSNYPLTFGGGTRLEIKRTVAAPSVFIFPPSDEQLKSGTASVVCLLNNFYPREAKVQWKVDNALQSGNSQESVTEQDSKDSTYSLSSTLTLSKADYEKHKVYACEVTHQGLSSPVTKSFNRGEC

SEQ ID NO: 39 - protein, 215 aa, Homo sapiens
EIVLTQSPSSLSASVGDRVTITCRASQGIGDDLGWYQQKPGKAPILLIYGTSTLQSGVPSRFSGSGSGTDFTLTINSLQPEDFATYYCLQDSNYPLTFGGGTRLEIKGRTVAAPSVFIFPPSDEQLKSGTASVVCLLNNFYPREAKVQWKVDNALQSGNSQESVTEQDSKDSTYSLSSTLTLSKADYEKHKVYACEVTHQGLSSPVTKSFNRGEC

SEQ ID NO: 40 - protein, 216 aa, Homo sapiens
EIVLTQSPSSLSASVGDRVTITCRASQGIGDDLGWYQQKPGKAPILLIYGTSTLQSGVPSRFSGSGSGTDFTLTINSLQPEDFATYYCLQDSNYPLTFGGGTRLEIKGGRTVAAPSVFIFPPSDEQLKSGTASVVCLLNNFYPREAKVQWKVDNALQSGNSQESVTEQDSKDSTYSLSSTLTLSKADYEKHKVYACEVTHQGLSSPVTKSFNRGEC

SEQ ID NO: 41 - protein, 217 aa, Homo sapiens
EIVLTQSPSSLSASVGDRVTITCRASQGIGDDLGWYQQKPGKAPILLIYGTSTLQSGVPSRFSGSGSGTDFTLTINSLQPEDFATYYCLQDSNYPLTFGGGTRLEIKGGSRTVAAPSVFIFPPSDEQLKSGTASVVCLLNNFYPREAKVQWKVDNALQSGNSQESVTEQDSKDSTYSLSSTLTLSKADYEKHKVYACEVTHQGLSSPVTKSFNRGEC

SEQ ID NO: 42 - protein, 218 aa, Homo sapiens
EIVLTQSPSSLSASVGDRVTITCRASQGIGDDLGWYQQKPGKAPILLIYGTSTLQSGVPSRFSGSGSGTDFTLTINSLQPEDFATYYCLQDSNYPLTFGGGTRLEIKGGGSRTVAAPSVFIFPPSDEQLKSGTASVVCLLNNFYPREAKVQWKVDNALQSGNSQESVTEQDSKDSTYSLSSTLTLSKADYEKHKVYACEVTHQGLSSPVTKSFNRGEC

SEQ ID NO: 43 - protein, 219 aa, Homo sapiens
EIVLTQSPSSLSASVGDRVTITCRASQGIGDDLGWYQQKPGKAPILLIYGTSTLQSGVPSRFSGSGSGTDFTLTINSLQPEDFATYYCLQDSNYPLTFGGGTRLEIKGGGGSRTVAAPSVFIFPPSDEQLKSGTASVVCLLNNFYPREAKVQWKVDNALQSGNSQESVTEQDSKDSTYSLSSTLTLSKADYEKHKVYACEVTHQGLSSPVTKSFNRGEC

SEQ ID NO: 44 - protein, 8 aa, Homo sapiens
TVTVSSAS

SEQ ID NO: 45 - protein, 9 aa, Homo sapiens
TVTVSGSAS

SEQ ID NO: 46 - protein, 10 aa, Homo sapiens
TVTVSGGSAS

SEQ ID NO: 47 - protein, 9 aa, Homo sapiens
TVTVSGGSA

SEQ ID NO: 48 - protein, 13 aa, Homo sapiens
TVTVSGGGGSSAS

SEQ ID NO: 49 - DNA, 738 bp, Homo sapiens
atgggctggtcctgcatcatcctgtttctggtggccaccgccaccggcgtgcactctgaagtgcagctggtggaatctggcggcggagtggtgcagcctggcagaagcctgagactgagctgtgccgccagcggcttcaccttcagcagctacggaatgcactgggtgcgccaggcccctggcaaagaactggaatgggtggccgtgatcagctacgacggcagcatcaagtactacgccgacagcgtgaagggccggttcaccatctcccgggacaacagcaagaacaccctgtacctgcagatgaacagcctgcgggccgaggacaccgccgtgtactactgtgctagaaccggcgagtacagcggctacgacaccgaccctcagtactcttggggccagggcaccaccgtgacagtgtctagcgccagcaccaagggcccaagcgtgttccctctggccccttgcagcagaagcaccagcgaatctacagccgccctgggctgcctcgtgaaggactactttcccgagcccgtgacagtgtcctggaactctggcgccctgaccagcggagtgcatacctttccagccgtgctgcagagcagcggcctgtactctctgagcagcgtcgtgactgtgcccagcagctctctgggcaccaagacctacacctgtaacgtggaccacaagcccagcaacaccaaggtggacaagagagtgcatcaccaccaccatcac

SEQ ID NO: 50 - DNA, 29 bp, Homo sapiens
ccaccgtgacagtgtctggcagcgccagc

SEQ ID NO: 51 - DNA, 29 bp, Homo sapiens
gctggcgctgccagacactgtcacggtgg

SEQ ID NO: 52 - DNA, 32 bp, Homo sapiens
ccaccgtgacagtgtctggcggcagcgccagc

SEQ ID NO: 53 - DNA, 32 bp, Homo sapiens
gctggcgctgccgccagacactgtcacggtgg

SEQ ID NO: 54 - DNA, 44 bp, Homo sapiens
caccaccgtgacagtgtctggcggcggcggcagcagcgccagca

SEQ ID NO: 55 - DNA, 44 bp, Homo sapiens
tgctggcgctgctgccgccgccgccagacactgtcacggtggtg

SEQ ID NO: 56 - protein, 454 aa, Homo sapiens
EVQLVESGGGVVQPGRSLRLSCAASGFTFSSYGMHWVRQAPGKELEWVAVISYDGSIKYYADSVKGRFTISRDNSKNTLYLQMNSLRAEDTAVYYCARTGEYSGYDTDPQYSWGQGTTVTVSGSASTKGPSVFPLAPSSKSTSGGTAALGCLVKDYFPEPVTVSWNSGALTSGVHTFPAVLQSSGLYSLSSVVTVPSSSLGTQTYICNVNHKPSNTKVDKKVEPKSCDKTHTCPPCPAPELLGGPSVFLFPPKPKDTLMISRTPEVTCVVVDVSHEDPEVKFNWYVDGVEVHNAKTKPREEQYNSTYRVVSVLTVLHQDWLNGKEYKCKVSNKALPAPIEKTISKAKGQPREPQVYTLPPSRDELTKNQVSLTCLVKGFYPSDIAVEWESNGQPENNYKTTPPVLDSDGSFFLYSKLTVDKSRWQQGNVFSCSVMHEALHNHYTQKSLSLSPGK

SEQ ID NO: 57 - protein, 453 aa, Homo sapiens
EVQLVESGGGVVQPGRSLRLSCAASGFTFSSYGMHWVRQAPGKELEWVAVISYDGSIKYYADSVKGRFTISRDNSKNTLYLQMNSLRAEDTAVYYCARTGEYSGYDTDPQYSWGQGTTVTVSGGSAKGPSVFPLAPSSKSTSGGTAALGCLVKDYFPEPVTVSWNSGALTSGVHTFPAVLQSSGLYSLSSVVTVPSSSLGTQTYICNVNHKPSNTKVDKKVEPKSCDKTHTCPPCPAPELLGGPSVFLFPPKPKDTLMISRTPEVTCVVVDVSHEDPEVKFNWYVDGVEVHNAKTKPREEQYNSTYRVVSVLTVLHQDWLNGKEYKCKVSNKALPAPIEKTISKAKGQPREPQVYTLPPSRDELTKNQVSLTCLVKGFYPSDIAVEWESNGQPENNYKTTPPVLDSDGSFFLYSKLTVDKSRWQQGNVFSCSVMHEALHNHYTQKSLSLSPGK

SEQ ID NO: 58 - protein, 458 aa, Homo sapiens
EVQLVESGGGVVQPGRSLRLSCAASGFTFSSYGMHWVRQAPGKELEWVAVISYDGSIKYYADSVKGRFTISRDNSKNTLYLQMNSLRAEDTAVYYCARTGEYSGYDTDPQYSWGQGTTVTVSGGGGSSASTKGPSVFPLAPSSKSTSGGTAALGCLVKDYFPEPVTVSWNSGALTSGVHTFPAVLQSSGLYSLSSVVTVPSSSLGTQTYICNVNHKPSNTKVDKKVEPKSCDKTHTCPPCPAPELLGGPSVFLFPPKPKDTLMISRTPEVTCVVVDVSHEDPEVKFNWYVDGVEVHNAKTKPREEQYNSTYRVVSVLTVLHQDWLNGKEYKCKVSNKALPAPIEKTISKAKGQPREPQVYTLPPSRDELTKNQVSLTCLVKGFYPSDIAVEWESNGQPENNYKTTPPVLDSDGSFFLYSKLTVDKSRWQQGNVFSCSVMHEALHNHYTQKSLSLSPGK

SEQ ID NO: 59 - DNA, 35 bp, Homo sapiens
caccaccgtgacagtgtctggcggcagcgccagca

SEQ ID NO: 60 - DNA, 35 bp, Homo sapiens
tgctggcgctgccgccagacactgtcacggtggtg

SEQ ID NO: 61 - protein, 455 aa, Homo sapiens
EVQLVESGGGVVQPGRSLRLSCAASGFTFSSYGMHWVRQAPGKELEWVAVISYDGSIKYYADSVKGRFTISRDNSKNTLYLQMNSLRAEDTAVYYCARTGEYSGYDTDPQYSWGQGTTVTVSGGSASTKGPSVFPLAPSSKSTSGGTAALGCLVKDYFPEPVTVSWNSGALTSGVHTFPAVLQSSGLYSLSSVVTVPSSSLGTQTYICNVNHKPSNTKVDKKVEPKSCDKTHTCPPCPAPELLGGPSVFLFPPKPKDTLMISRTPEVTCVVVDVSHEDPEVKFNWYVDGVEVHNAKTKPREEQYNSTYRVVSVLTVLHQDWLNGKEYKCKVSNKALPAPIEKTISKAKGQPREPQVYTLPPSRDELTKNQVSLTCLVKGFYPSDIAVEWESNGQPENNYKTTPPVLDSDGSFFLYSKLTVDKSRWQQGNVFSCSVMHEALHNHYTQKSLSLSPGK